European Patent Application EP 4 537 840 A1, published April 16, 2025. Title: Soluble HCV glycorotein E2 as a vaccine against Hepatitis C virus. Applicant: Twincore Zentrum für Experimentelle und Klinische Infektionsforschung GmbH. The sequence listing filed with the application follows.

SEQUENCE LISTING (13 sequences)

SEQ ID NO: 1 - protein, 332 aa, Hepatitis C virus
ETHVSGAAVGRSTAGLANLFSSGSKQNLQLINSNGSWHINRTALNCNDSLNTGFLASLFYTHKFNSSGCSERLACCKSLDSYGQGWGPLGVANISGSSDDRPYCWHYAPRPCGIVPASSVCGPVYCFTPSPVVVGTTDHVGVPTYTWGENETDVFLLNSTRPPHGAWFGCVWMNSTGFTKTCGAPPCEVNTNNGTWHCPTDCFRKHPETTYAKCGSGPWITPRCLIDYPYRLWHFPCTANFSVFNIRTFVGGIEHRMQAACNWTRGEVCGLEHRDRVELSPLLLTTTAWQILPCSFTTLPALSTGLIHLHQNIVDVQYLYGVGSAVVSWALK

SEQ ID NO: 2 - protein, 336 aa, Hepatitis C virus
TTYSSGQEAGRTVLGFTNLFTSGAKQNLYLINTNGSWHINRTALNCNDSLQTGFMASLFYTHRFNSSGCPERLSSCRGLDDFRIGWGTLEYETHVTNDEDMRPYCWHYPPRPCGIVPARTVCGPVYCFTPSPVVVGTTDKQGVPTYTWGENETDVFLLNSTRPPRGAWFGCTWMNGTGFTKTCGAPPCRIRKDYNSTIDLLCPTDCFRKHPDATYLKCGAGPWLTPRCLVDYPYRLWHYPCTVNFTIFKARMYVGGVEHRFSAACNFTRGDRCRLEDRDRGQQSPLLHSTTEWAVLPCSFSDLPALSTGLLHLHQNIVDVQYLYGLSPALTRYIVK

SEQ ID NO: 3 - protein, 336 aa, Hepatitis C virus
NTYSSGAQAGRTTSVLTSLFTSGPQQRINLVNTNGSWHINRTALNCNDSLQTGFIASLFYTHKFNSSGCPERLSSCRTLDDFRIGWGALEYETNVTNDDDMRPYCWHYPPKPCGIVSARTVCGPVYCFTPSPVVVGTTDRQGVPTYSWGENETDVFLLNSTRPPRGAWFGCTWMNGTGFTKTCGAPPCRIRGDFNATLDLLCPTDCFRKHPDTTYLRCGSGPWLTPRCLVEYPYRLWHYPCTVNFTISKVRMYVGGVEHRFSAACNFTRGDRCGLEDRDRGQQSPLLHSTTEWAVLPCSFSDLPALSTGLLHLHQNIVDVQYLYGLSPALTRYIVK

SEQ ID NO: 4 - protein, 332 aa, Hepatitis C virus
ETHVTGGNAGRTTAGLVGLLTPGAKQNIQLINTNGSWHINSTALNCNESLNTGWLAGLFYQHKFNSSGCPERLASCRRLTDFAQGWGPISYANGSGLDERPYCWHYPPRPCGIVPAKSVCGPVYCFTPSPVVVGTTDRSGAPTYSWGANDTDVFVLNNTRPPLGNWFGCTWMNSTGFTKVCGAPPCVIGGVGNNTLLCPTDCFRKHPEATYSRCGSGPWITPRCMVDYPYRLWHYPCTINYTIFKVRMYVGGVEHRLEAACNWTRGERCDLEDRDRSELSPLLLSTTQWQVLPCSFTTLPALSTGLIHLHQNIVDVQYLYGVGSSIASWAIK

SEQ ID NO: 5 - protein, 338 aa, Hepatitis C virus
ETYVTGGSVAHSARGLTSLFSMGAKQKLQLVNTNGSWHINSTALNCNESINTGFIAGLFYYHKFNSTGCPQRLSSCKPIISFRQGWGPLTDANITGPSDDRPYCWHYAPRPCSVVPASSVCGPVYCFTPSPVVVGTTDIKGKPTYNWGENETDVFLLESLRPPSGRWFGCAWMNSTGFLKTCGAPPCNIYGGEGDPENETDLFCPTDCFRKHPEATYSRCGAGPWLTPRCMVDYPYRLWHYPCTVNFTLFKVRMFVGGFEHRFTAACNWTRGERCNIEDRDRSEQHPLLHSTTELAILPCSFTPMPALSTGLIHLHQNIVDVQYLYGVGSDMVGWALK

SEQ ID NO: 6 - protein, 336 aa, Hepatitis C virus
HTHVVGGSVAQGARGFTGLFSPGSQQNIQLINTNGSWHINRTALNCNDSLNTGFLASLFYTHKFNSSGCPERMSACKGIEAFRIGWGVLEHEENVTNDEDMRPYCWHYPPKPCGIVPARTVCGPVYCFTPSPVVVGTTDRRGVPTYTWGENETDVFLLNSTRPPGGSWFGCTWMNSTGYTKTCGAPPCRIRADFNASTDLLCPTDCFRKHPDATYGKCGAGPWLTPKCLVDYPYRLWHYPCTVNFTIFKIRMYVGGVEHRLQAACNFSRGDRCNLEDRDRSQLSPLLHSTTEWAILPCTFSDMPALSTGLLHLHQNIVDVQYLYGLSPALTKYMVK

SEQ ID NO: 7 - protein, 336 aa, Hepatitis C virus
RTHITGAHVGRTASSLASLFNSGPQQRLSLINTNGSWHINRTALNCNDSLQTGFITALFYSKHFNSSGCPERLSSCRGLDDFRIGWGPLEYETNVTNGEDMRPYCWHYPPKPCGIVSAKTVCGPVYCFTPSPVVVGTTDKQGVPTYSWGENETDVFLLNSTRPPQGAWFGCTWMNGTGYTKTCGAPPCRIRRDYNGTLDLLCPTDCFRKHPDTTYLKCGAGPWLTPKCLVDYPYRLWHYPCTVNFTIHKVRMYVGGVEHRLNAACNFTRGDRCRLDDRDRGQQSPLLHSTTEWAVLPCTFSDLPALSTGLLHLHQNIVDVQYLYGLSPAITRYIVK

SEQ ID NO: 8 - protein, 332 aa, Hepatitis C virus
ETHTTGRVAGHTTSGFTSLFSSGASQKIQLVNTNGSWHINRTALNCNDSLQTGFFAALFYAHKFNSSGCPERMASCRPIDWFAQGWGPITYTKPNSSDQRPYCWHYAPRPCGVVPASQVCGPVYCFTPSPVVVGTTDRSGVPTYSWGENETDVMLLNNTRPPQGNWFGCTWMNSTGFTKTCGGPPCNIGGVGNRTLICPTDCFRKHPEATYTKCGSGPWLTPRCLVDYPYRLWHYPCTLNFSIFKVRMYVGGVEHRLNAACNWTRGERCNLEDRDRSELSPLLLSTTEWQILPCAFTTLPALSTGLIHLHQNIVDVQYLYGVGSAFVSFAIK

SEQ ID NO: 9 - protein, 333 aa, Hepatitis C virus
STRTVGGSAAQGARGLASLFTPGPQQNLQLINTNGSWHINRTALNCNDSLQTGFVAGLLYYHKFNSTGCPQRMASCRPLAAFDQGWGTISYAAVSGPSDDKPYCWHYPPRPCGIVPARGVCGPVYCFTPSPVVVGTTDRKGNPTYSWGENETDIFLLNNTRPPTGNWFGCTWMNSTGFVKTCGAPPCNLGPTGNNSLKCPTDCFRKHPDATYTKCGSGPWLTPRCLVHYPYRLWHYPCTLNYTIFKVRMYIGGLEHRLEVACNWTRGERCDLEDRDRAELSPLLHTTTQWAILPCSFTPTPALSTGLIHLHQNIVDTQYLYGLSSSIVSWAVK

SEQ ID NO: 10 - protein, 336 aa, Hepatitis C virus
RTHTVGGSAAQTTGRLTSLFDMGPRQKIQLVNTNGSWHINRTALNCNDSLHTGFIASLFYTHSFNSSGCPERMSACRSIEAFRVGWGALQYEDNVTNPEDMRPYCWHYPPRQCGVVSAKTVCGPVYCFTPSPVVVGTTDRLGAPTYTWGENETDVFLLNSTRPPLGSWFGCTWMNSSGYTKTCGAPPCRTRADFNASTDLLCPTDCFRKHPDTTYLKCGSGPWLTPRCLIDYPYRLWHYPCTVNYTIFKIRMYVGGVEHRLTAACNFTRGDRCNLEDRDRSQLSPLLHSTTEWAILPCSYSDLPALSTGLLHLHQNIVDVQFMYGLSPALTKYIVR

SEQ ID NO: 11 - protein, 337 aa, Hepatitis C virus
QTRTIASSVASQASSLVGVFSSGPKQNIQLINTNGSWHINRHWPLTAMTPCNTGFIAALVYRNRFNSSGCPERLSACRNIESFRIGWGTLQYENNVTNSEDMRPYCWHYPPKQCDIVPARSVCGPVYCFTPSPIVVGTTDRLGVPTYTWGENETDVFLLNSTRPPRGSWFGCTWMNSSGFTKTCGAPPCRIRADFNASTDLLCPTDCFRKHPDATYIKCGSGPWLTPRCLVDYPYRLWHYPCTVNFTIFKIRMYVGGVEHRLTAACNFTRGDRCNLEDRDRSQLSPLLHSTTEWAILPCTFSDLPALSTGLLHLHQNIVDVQYMYGLSPALTKYVVR

SEQ ID NO: 12 - protein, 336 aa, Hepatitis C virus
QTHTISGHAARTTHGLVSLFTPGSQQNIQLVNTNGSWHINRTALNCNDSLKTGFIAALFYSHKFNSSGCPQRMSSCRSIEEFRIGWGNLEYEENVTNDDNMRPYCWHYPPRPCGIVPAQTVCGPVYCFTPSPVVVGTTDRRGVPTYTWGENDTDVFLLNSTRPPRGAWFGCTWMNSTGFTKTCGAPPCRIRPDFNSSEDLLCPTDCFRKHSEATYTRCGAGPWLTPKCLFHYPYRLWHYPCTINFTIHKIRMFIGGVEHRLEAACNFTRGDRCNLEDRDRSQLSPLLHSTTEWAILPCTFSDMPALSTGLLHLHQNIVDVQYLYGLSPAITKYIVK

SEQ ID NO: 13 - protein, 332 aa, Hepatitis C virus
GTYVTGGTMAKNTLGITSLFSPGSSQKIQLVNTNGSWHINRTALNCNDSLNTGFLAALFYVHKFNSSGCPERMASCSPIDAFAQGWGPITYNESHSSDQRPYCWHYAPRPCGIVPAAQVCGPVYCFTPSPVVVGTTDRFGVPTYSWGENETDVLLLNNTRPPQGNWFGCTWMNSTGFTKTCGGPPCNIGGIGNKTLTCPTDCFRKHPEATYTKCGSGPWLTPRCLVHYPYRLWHYPCTVNFTIFKVRMYVGGVEHRLEAACNWTRGERCNLEDRDRSELSPLLLSTTEWQVLPCSFTTLPALSTGLIHLHQNVVDVQYLYGIGSAVVSFAIK